European Patent Application EP 4 338 764 A2, published March 20, 2024. Title: Tissue Scaffold. Applicant: RAFT Enterprises Ltd. Application EP 23169720.2, filed July 13, 2018. The sequence listing filed with the application follows.

SEQUENCE LISTING (17 sequences)

SEQ ID NO: 1 - DNA, 21 bp, synthetic construct
  misc_feature 1..21: note = Synthetic primer
  source 1..21: mol_type = other DNA
cgcctgagcaaagtaaatgag

SEQ ID NO: 2 - DNA, 19 bp, synthetic construct
  misc_feature 1..19: note = Synthetic primer
  source 1..19: mol_type = other DNA
gccctcgatatagcggatg

SEQ ID NO: 3 - DNA, 25 bp, synthetic construct
  misc_feature 1..25: note = Synthetic primer
  source 1..25: mol_type = other DNA
gaataaagatggggttctcatatcc

SEQ ID NO: 4 - DNA, 21 bp, synthetic construct
  misc_feature 1..21: note = Synthetic primer
  source 1..21: mol_type = other DNA
aacttcagcaaactcaaactt

SEQ ID NO: 5 - DNA, 25 bp, synthetic construct
  misc_feature 1..25: note = Synthetic primer
  source 1..25: mol_type = other DNA
cggcaactctagtatttaggataac

SEQ ID NO: 6 - DNA, 24 bp, synthetic construct
  misc_feature 1..24: note = Synthetic primer
  source 1..24: mol_type = other DNA
caaataaaatgacaaggcacgatt

SEQ ID NO: 7 - DNA, 20 bp, synthetic construct
  misc_feature 1..20: note = Synthetic primer
  source 1..20: mol_type = other DNA
ttctccccttttcccactga

SEQ ID NO: 8 - DNA, 25 bp, synthetic construct
  misc_feature 1..25: note = Synthetic primer
  source 1..25: mol_type = other DNA
caaacgcaatcactatctataccat

SEQ ID NO: 9 - DNA, 19 bp, synthetic construct
  misc_feature 1..19: note = Synthetic primer
  source 1..19: mol_type = other DNA
ggaccagtacccgcacttg

SEQ ID NO: 10 - DNA, 20 bp, synthetic construct
  misc_feature 1..20: note = Synthetic primer
  source 1..20: mol_type = other DNA
aatccgggtggtccttcttg

SEQ ID NO: 11 - DNA, 23 bp, synthetic construct
  misc_feature 1..23: note = Synthetic primer
  source 1..23: mol_type = other DNA
cactaaggaaggaattgggaaca

SEQ ID NO: 12 - DNA, 25 bp, synthetic construct
  misc_feature 1..25: note = Synthetic primer
  source 1..25: mol_type = other DNA
gggattaaaatcaagagcatcattg

SEQ ID NO: 13 - DNA, 18 bp, synthetic construct
  misc_feature 1..18: note = Synthetic primer
  source 1..18: mol_type = other DNA
cgtttcgtgtccctttca

SEQ ID NO: 14 - DNA, 25 bp, synthetic construct
  misc_feature 1..25: note = Synthetic primer
  source 1..25: mol_type = other DNA
cctcttgttcattcttgttcgtatt

SEQ ID NO: 15 - protein, 5 aa, unidentified
GVGVP

SEQ ID NO: 16 - protein, 5 aa, unidentified
GVPGV

SEQ ID NO: 17 - protein, 6 aa, unidentified
GVGVAP